European Patent Application EP 4 782 004 A1, published July 29, 2026. Title: Gluten degrading protein and uses thereof. Applicant: Consejo Superior de Investigaciones Cientificas. The sequence listing filed with the application follows.

SEQUENCE LISTING (14 sequences)

SEQ ID NO: 1 - protein, 380 aa, synthetic construct
  source 1..380: organism (original language) = constructo sintetico
MQAKFFTFVILSSVFYFNYPLAEARSIQARLANKPKGTIKTIKGDDGEVVDCVDIYKQPAFDHPLLKNHTLQMQPSSYASKVGEYNKLEQPWHKNGECPKGSIPIRRQVITGLPVVKKQFPNLKFAPPSANTNHQYAVIAYFYGNASLQGANATINIWEPNLKNPNGDFSLTQIWISAGSGSSLNTIEAGWQVYPGRTGDSQPRFFIYWTADGYTSTGCYDLTCPGFVQTNNYYAIGMALQPSVYGGQQYELNESIQRDPATGNWWLYLWGTVVGYWPASIYNSITNGADTVEWGGEIYDSSGTGGFHTTTQMGSGHFPTEGYGKASYVRDLQVVDTYGNVISPTANSFQGIAPAPNCYNYQFQQGSSELYLFYGGPGCQ

SEQ ID NO: 2 - protein, 380 aa, synthetic construct
  source 1..380: organism (original language) = constructo sintetico
MQAKFFTFVILSSVFYFNYPLAEARSIQARLANKPKGTIKTIKGDDGEVVDCVDIYKQPAFDHPLLKNHTLQMQPSSYASKVGEYNKLEQPWHKNGECPKGSIPIRRQVITGLPVVKKQFPNLKFAPPSANTNHQYAVIAYFYGNASLQGANATINIWEPNLKNPNGDFSLTQIWISAGSGSSLNTIEAGWQVYPGRTGDSQPRFFIYWTADGYTSTGCYDLTCPGFVQTNNYYAIGMALQPSVYGGQQYELNESIQRDPATGNWWLYLWGTVVGYWPASIYNSITNGADTVEWGGEIYDSSGTGGFHTTTQMGSGHFPTEGYGKASYVRDLQCVDTYGNVISPTANSFQGIAPAPNCYNYQFQQGSSELYLFYGGPGCQ

SEQ ID NO: 3 - protein, 4 aa, synthetic construct
  source 1..4: organism (original language) = constructo sintetico
QPQL

SEQ ID NO: 4 - protein, 33 aa, synthetic construct
  source 1..33: organism (original language) = constructo sintetico
LQLQPFPQPQLPYPQPQLPYPQPQLPYPQPQPF

SEQ ID NO: 5 - protein, 9 aa, synthetic construct
  source 1..9: organism (original language) = constructo sintetico
AIAHHHHHH

SEQ ID NO: 6 - protein, 389 aa, synthetic construct
  source 1..389: organism (original language) = constructo sintetico
MQAKFFTFVILSSVFYFNYPLAEARSIQARLANKPKGTIKTIKGDDGEVVDCVDIYKQPAFDHPLLKNHTLQMQPSSYASKVGEYNKLEQPWHKNGECPKGSIPIRRQVITGLPVVKKQFPNLKFAPPSANTNHQYAVIAYFYGNASLQGANATINIWEPNLKNPNGDFSLTQIWISAGSGSSLNTIEAGWQVYPGRTGDSQPRFFIYWTADGYTSTGCYDLTCPGFVQTNNYYAIGMALQPSVYGGQQYELNESIQRDPATGNWWLYLWGTVVGYWPASIYNSITNGADTVEWGGEIYDSSGTGGFHTTTQMGSGHFPTEGYGKASYVRDLQCVDTYGNVISPTANSFQGIAPAPNCYNYQFQQGSSELYLFYGGPGCQAIAHHHHHH

SEQ ID NO: 7 - protein, 380 aa, synthetic construct
  source 1..380: organism (original language) = constructo sintetico
MQAKFFTFVILSSVFYFNYPLAEAKTLNAELSNKPRGTIKSIKGDDGEMVDCVDIYKQPAFDHPKLKNPSLQMQPNSYASKVGEYNKLKQSWHKSGECPEVSIPIRRQVISGVPVVRKQFPNLKFAPPSANTNHQYAVIAYFYGNASLQGANATINIWEPTLKNPDKDFSLTQIWISAGSGTNLNTIEAGWQVYPGRTGDSQPRFFIYWTADGYSSSGCYDLTCPGFVQVNNYYAIGMALKPSTYGAEQYELNESIQRDPATGNWWLYLWSVVVGYWPSSIYNTITEGADTVEWGGEIYDSSGSGGYHTTTQMGSGHFPREGYGRASYVRDLQVTDERGQTITPPTEKFQGIAPAPQCYKYEFQEGKKELYLFYGGPGCQ

SEQ ID NO: 8 - protein, 380 aa, synthetic construct
  source 1..380: organism (original language) = constructo sintetico
MQAKFFTFVILSSVFYFNYPLAEAKTLNAELSNKPRGTIKSIKGDDGEMVDCVDIYKQPAFDHPKLKNPSLQMQPNSYASKVGEYNKLKQSWHKSGECPEVSIPIRRQVISGVPVVRKQFPNLKFAPPSANTNHQYAVIAYFYGQASLQGATATINIWEPTLKNPDKDFSLTQIWISAGSGTNLNTIEAGWQVYPGRTGDSQPRFFIYWTADGYSSSGCYDLTCPGFVQVNNYYAIGMALKPSTYGAEQYELNESIQRDPATGNWWLYLWSVVVGYWPSSIYNTITEGADTVEWGGEIYDSSGSGGYHTTTQMGSGHFPREGYGRASYVRDLQVTDERGQTITPPTEKFQGIAPAPQCYKYEFQEGKKELYLFYGGPGCQ

SEQ ID NO: 9 - protein, 380 aa, synthetic construct
  source 1..380: organism (original language) = constructo sintetico
MQAKFFTFVILSSVFYFNYPLAEARSIQARLANKPKGTIKTIKGDDGEVVDCVDIYKQPAFDHPLLKNHTLQMQPSSYASKVGEYNKLEQPWHKNGECPKGSIPIRRQVITGLPVVKKQFPNLKFAPPSANTNHQYAVIAYFYGQASLQGANATINIWEPNLKNPNGDFSLTQIWISAGSGSSLNTIEAGWQVYPGRTGDSQPRFFIYWTADGYTSTGCYDLTCPGFVQTNNYYAIGMALQPSVYGGQQYELNESIQRDPATGNWWLYLWGTVVGYWPASIYNSITNGADTVEWGGEIYDSSGTGGFHTTTQMGSGHFPTEGYGKASYVRDLQVVDTYGNVISPTANSFQGIAPAPNCYNYQFQQGSSELYLFYGGPGCQ

SEQ ID NO: 10 - protein, 380 aa, synthetic construct
  source 1..380: organism (original language) = constructo sintetico
MQAKFFTFVILSSVFYFNYPLAEARSIQARLANKPKGTIKTIKGDDGEVVDCVDIYKQPAFDHPLLKNHTLQMQPSSYASKVGEYNKLEQPWHKNGECPKGSIPIRRQVITGLPVVKKQFPNLKFAPPSANTNHQYAVIAYFYGNASLQGATATINIWEPNLKNPNGDFSLTQIWISAGSGSSLNTIEAGWQVYPGRTGDSQPRFFIYWTADGYTSTGCYDLTCPGFVQTNNYYAIGMALQPSVYGGQQYELNESIQRDPATGNWWLYLWGTVVGYWPASIYNSITNGADTVEWGGEIYDSSGTGGFHTTTQMGSGHFPTEGYGKASYVRDLQVVDTYGNVISPTANSFQGIAPAPNCYNYQFQQGSSELYLFYGGPGCQ

SEQ ID NO: 11 - protein, 380 aa, synthetic construct
  source 1..380: organism (original language) = constructo sintetico
MQAKFFTFVILSSVFYFNYPLAEARSIQARLANKPKGTIKTIKGDDGEVVDCVDIYKQPAFDHPLLKNHTLQMQPSSYASKVGEYNKLEQPWHKNGECPKGSIPIRRQVITGLPVVKKQFPNLKFAPPSANTNHQYAVIAYFYGQASLQGATATINIWEPNLKNPNGDFSLTQIWISAGSGSSLNTIEAGWQVYPGRTGDSQPRFFIYWTADGYTSTGCYDLTCPGFVQTNNYYAIGMALQPSVYGGQQYELNESIQRDPATGNWWLYLWGTVVGYWPASIYNSITNGADTVEWGGEIYDSSGTGGFHTTTQMGSGHFPTEGYGKASYVRDLQVVDTYGNVISPTANSFQGIAPAPNCYNYQFQQGSSELYLFYGGPGCQ

SEQ ID NO: 12 - DNA, 1068 bp, synthetic construct
  source 1..1068: mol_type = other DNA; organism (original language) = constructo sintetico
cgtagcattcaggcgcgtctggcgaataaaccgaaaggcaccatcaaaaccatcaagggcgacgacggcgaagttgtggattgcgttgacatctacaagcagccggcgttcgatcacccgctgctgaaaaaccacaccctgcagatgcaaccgagcagctatgcgagcaaggttggcgagtacaacaaactggaacaaccgtggcacaagaacggcgagtgcccgaaaggcagcatcccgattcgtcgtcaggtgatcaccggtctgccggtggttaagaaacaattcccgaacctgaagtttgctccgccgagcgcgaacaccaaccaccagtatgcggttattgcgtacttctatggtaacgcgagcctgcaaggcgcgaacgcgaccatcaacatttgggagccgaacctgaaaaacccgaacggtgactttagcctgacccagatctggattagcgcgggtagcggcagcagcctgaacaccattgaagcgggttggcaggtgtatccgggtcgtaccggtgatagccaaccgcgtttctttatttactggaccgcggacggttataccagcaccggctgctacgatctgacctgcccgggtttcgttcagaccaacaactactatgcgatcggcatggcgctgcaaccgagcgtgtacggtggccagcaatatgagctgaacgaaagcattcagcgtgacccggcgaccggtaactggtggctgtatctgtggggtaccgtggttggctattggccggcgagcatctacaacagcattaccaacggtgcggacaccgttgagtggggtggcgaaatctacgatagcagcggtaccggtggcttccacaccaccacccaaatgggtagcggccactttccgaccgaaggttacggcaaggcgagctatgtgcgtgacctgcagtgcgttgatacctatggtaacgtgatcagcccgaccgcgaacagctttcaaggcattgcgccggcgccgaactgctacaactatcaatttcagcagggcagcagcgaactgtacctgttttacggtggtccgggttgccaa

SEQ ID NO: 13 - DNA, 27 bp, synthetic construct
  source 1..27: mol_type = other DNA; organism (original language) = constructo sintetico
gtgacctgcaggtcgttgatacctatg

SEQ ID NO: 14 - DNA, 21 bp, synthetic construct
  source 1..21: mol_type = other DNA; organism (original language) = constructo sintetico
gcacatagctcgccttgccgt